European Patent Application EP 4 230 652 A1, published August 23, 2023. Title: Anti-OSCAR antibody for prevention or treatment of osteoarthritis. Applicant: Ewha University - Industry Collaboration Foundation. The sequence listing filed with the application follows.

SEQUENCE LISTING (29 sequences)

SEQ ID NO: 1 - DNA, 19 bp, Artificial Sequence
  pC3X-f
gcacgacaggtttcccgac

SEQ ID NO: 2 - DNA, 20 bp, Artificial Sequence
  pC3X-b
aaccatcgatagcagcaccg

SEQ ID NO: 3 - DNA, 22 bp, Artificial Sequence
  ompseq
aagacagctatcgcgattgcag

SEQ ID NO: 4 - protein, 477 aa, Artificial Sequence
  hOSCAR-Fc
METDTLLLWVLLLWVPGSTGDITPSVAIIVPPASYHPKPWLGAQPATVVTPGVNVTLRCRAPQPAWRFGLFKPGEIAPLLFRDVSSELAEFFLEEVTPAQGGSYRCCYRRPDWGPGVWSQPSDVLELLVTEELPRPSLVALPGPVVGPGANVSLRCAGRLRNMSFVLYREGVAAPLQYRHSAQPWADFTLLGARAPGTYSCYYHTPSAPYVLSQRSEVLVISWEDSGSSDYTRGNLVRLGLAGLVGQAGQEPKSSDKTHTCPPCPAPELLGGPSVFLFPPKPKDTLMISRTPEVTCVVVDVSHEDPEVKFNWYVDGVEVHNAKTKPREEQYNSTYRVVSVLTVLHQDWLNGKEYKCKVSNKALPAPIEKTISKAKGQPREPQVYTLPPSRDELTKNQVSLTCLVKGFYPSDIAVEWESNGQPENNYKTTPPVLDSDGSFFLYSKLTVDKSRWQQGNVFSCSVMHEALHNHYTQKSLS

SEQ ID NO: 5 - protein, 462 aa, Artificial Sequence
  mOSCAR-Fc
METDTLLLWVLLLWVPGSTGDFTPTAPLASYPQPWLGAHPAAVVTPGINVTLTCRAPQSAWRFALFKSGLVTPLLLRDVSVELAEFFLEEVTPAQGGSYHCRYRKTDWGPGVWSQPSNVLELLVTDQLPRPSLVALPGPVVAPGANVSLRCAGRIPGMSFALYRVGVATPLQYIDSVQPWADFLLIGTHTPGTYCCYYHTPSAPYVLSQRSQPLVISFEGSGSLDYTQGNGQAGQEPKSSDKTHTCPPCPAPELLGGPSVFLFPPKPKDTLMISRTPEVTCVVVDVSHEDPEVKFNWYVDGVEVHNAKTKPREEQYNSTYRVVSVLTVLHQDWLNGKEYKCKVSNKALPAPIEKTISKAKGQPREPQVYTLPPSRDELTKNQVSLTCLVKGFYPSDIAVEWESNGQPENNYKTTPPVLDSDGSFFLYSKLTVDKSRWQQGNVFSCSVMHEALHNHYTQKSLS

SEQ ID NO: 6 - protein, 116 aa, Artificial Sequence
  B4_VH_AA
EVQLLESGGGLVQPGGSLRLSCAASGFTFSDYAMSWVRQAPGKGLEWVSGIYHGGGNIYYADSVKGRFTISRDNSKNTLYLQMNSLRAEDTAVYYCARAPDEFDYWGQGTLVTVSS

SEQ ID NO: 7 - protein, 110 aa, Artificial Sequence
  B4_VL_AA
QSVLTQPPSASGTPGQRVTISCSGSSSNIGNNSVTWYQQLPGTAPKLLIYYNSHRPSGVPDRFSGSKPGTSASLAISGLRSEDEADYYCGAWDSSLNGYVFGGGTKLTVL

SEQ ID NO: 8 - protein, 446 aa, Artificial Sequence
  B4_IGG-H_AA
EVQLLESGGGLVQPGGSLRLSCAASGFTFSDYAMSWVRQAPGKGLEWVSGIYHGGGNIYYADSVKGRFTISRDNSKNTLYLQMNSLRAEDTAVYYCARAPDEFDYWGQGTLVTVSSASTKGPSVFPLAPSSKSTSGGTAALGCLVKDYFPEPVTVSWNSGALTSGVHTFPAVLQSSGLYSLSSVVTVPSSSLGTQTYICNVNHKPSNTKVDKKVEPKSCDKTHTCPPCPAPELLGGPSVFLFPPKPKDTLMISRTPEVTCVVVDVSHEDPEVKFNWYVDGVEVHNAKTKPREEQYNSTYRVVSVLTVLHQDWLNGKEYKCKVSNKALPAPIEKTISKAKGQPREPQVYTLPPSRDELTKNQVSLTCLVKGFYPSDIAVEWESNGQPENNYKTTPPVLDSDGSFFLYSKLTVDKSRWQQGNVFSCSVMHEALHNHYTQKSLSLSPGK

SEQ ID NO: 9 - protein, 216 aa, Artificial Sequence
  B4_IGG-L_AA
QSVLTQPPSASGTPGQRVTISCSGSSSNIGNNSVTWYQQLPGTAPKLLIYYNSHRPSGVPDRFSGSKPGTSASLAISGLRSEDEADYYCGAWDSSLNGYVFGGGTKLTVLGQPKAAPSVTLFPPSSEELQANKATLVCLISDFYPGAVTVAWKADSSPVKAGVETTTPSKQSNNKYAASSYLSLTPEQWKSHKSYSCQVTHEGSTVEKTVAPAECS

SEQ ID NO: 10 - DNA, 348 bp, Artificial Sequence
  B4_VH_NT
gaggtgcagctgttggagtctgggggaggcttggtacagcctggggggtccctgagactctcctgtgcagcctctggattcacctttagcgattatgctatgagctgggtccgccaggctccagggaaggggctggagtgggtctcagggatctatcatggtggtggtaatatatattacgctgattctgtaaaaggtcggttcaccatctccagagacaattccaagaacacgctgtatctgcaaatgaacagcctgagagccgaggacacggccgtgtattactgtgcgagagctcctgatgagttcgactactggggccagggtacactagtcaccgtgagctca

SEQ ID NO: 11 - DNA, 330 bp, Artificial Sequence
  B4_VL_NT
cagtctgtgctgactcagccaccctcagcgtctgggacccccgggcagagggtcaccatctcttgtagtggctcttcatctaatattggcaataattctgtcacctggtaccagcagctcccaggaacggcccccaaactcctcatctattataatagtcatcggccaagcggggtccctgaccgattctctggctccaagcctggcacctcagcctccctggccatcagtgggctccggtccgaggatgaggctgattattactgtggtgcttgggattctagcctgaatggttatgtcttcggcggaggcaccaagctgacggtccta

SEQ ID NO: 12 - DNA, 1338 bp, Artificial Sequence
  B4_IGG-H_NT
gaggtgcagctgttggagtctgggggaggcttggtacagcctggggggtccctgagactctcctgtgcagcctctggattcacctttagcgattatgctatgagctgggtccgccaggctccagggaaggggctggagtgggtctcagggatctatcatggtggtggtaatatatattacgctgattctgtaaaaggtcggttcaccatctccagagacaattccaagaacacgctgtatctgcaaatgaacagcctgagagccgaggacacggccgtgtattactgtgcgagagctcctgatgagttcgactactggggccagggtacactagtcaccgtgagctcagctagcaccaagggcccatcggtcttccccctggcaccctcctccaagagcacctctgggggcacagcggccctgggctgcctggtcaaggactacttccccgaaccggtgacggtgtcgtggaactcaggcgccctgaccagcggcgtgcacaccttcccggctgtcctacagtcctcaggactctactccctcagcagcgtggtgaccgtgccctccagcagcttgggcacccagacctacatctgcaacgtgaatcacaagcccagcaacaccaaggtggacaagaaagttgagcccaaatcttgcgacaaaactcacacatgcccaccgtgcccagcacctgaactcctggggggaccgtcagtcttcctcttccccccaaaacccaaggacaccctcatgatctcccggacccctgaggtcacatgcgtggtggtggacgtgagccacgaagaccctgaggtcaagttcaactggtacgtggacggcgtggaggtgcataatgccaagacaaagccgcgggaggagcagtacaacagcacgtaccgtgtggtcagcgtcctcaccgtcctgcaccaggactggctgaatggcaaggagtacaagtgcaaggtctccaacaaagccctcccagcccccatcgagaaaaccatctccaaagccaaagggcagccccgagaaccacaggtgtacaccctgcccccatcccgggatgagctgaccaagaaccaggtcagcctgacctgcctggtcaaaggcttctatcccagcgacatcgccgtggagtgggagagcaatgggcagccggagaacaactacaagaccacgcctcccgtgctggactccgacggctccttcttcctctacagcaagctcaccgtggacaagagcaggtggcagcaggggaacgtcttctcatgctccgtgatgcatgaggctctgcacaaccactacacgcagaagagcctctccctgtccccgggtaaa

SEQ ID NO: 13 - DNA, 648 bp, Artificial Sequence
  B4_IGG-L_NT
cagtctgtgctgactcagccaccctcagcgtctgggacccccgggcagagggtcaccatctcttgtagtggctcttcatctaatattggcaataattctgtcacctggtaccagcagctcccaggaacggcccccaaactcctcatctattataatagtcatcggccaagcggggtccctgaccgattctctggctccaagcctggcacctcagcctccctggccatcagtgggctccggtccgaggatgaggctgattattactgtggtgcttgggattctagcctgaatggttatgtcttcggcggaggcaccaagctgacggtcctaggtcagcccaaggctgccccctcggtcacgctcttcccaccctcctctgaggagcttcaagccaacaaggccacactggtgtgtctcataagtgacttctacccgggagccgtgacagtggcctggaaggcagatagcagccccgtcaaggcgggagtggagaccaccacaccctccaaacaaagcaacaacaagtacgcggccagcagctacctgagcctgacgcctgagcagtggaagtcccacaaaagctacagctgccaggtcacgcatgaagggagcaccgtggagaagacagtggcccctgcagaatgctct

SEQ ID NO: 14 - protein, 118 aa, Artificial Sequence
  D11_VH_AA
EVQLLESGGGLVQPGGSLRLSCAASGFTFSDYYWTWVRQAPGKGLEWVSGSPVFGAANYAQNFQGRFTISRDNSKNTLYLQMNSLRAEDTAVYYCAKAGFTGGHFDIWGQGTLVTVSS

SEQ ID NO: 15 - protein, 108 aa, Artificial Sequence
  D11_VL_AA
QSVLTQPPSASGTPGQRVTISCSGSSSNIGNNYVSWYQQLPGTAPKLLIYGNSNRPSGVPNRFSGSKSGTSASLAISGLRSEDEADYYCQSYDSSSWLFGGGTKLTVL

SEQ ID NO: 16 - protein, 448 aa, Artificial Sequence
  D11_IGG-H_AA
EVQLLESGGGLVQPGGSLRLSCAASGFTFSDYYWTWVRQAPGKGLEWVSGSPVFGAANYAQNFQGRFTISRDNSKNTLYLQMNSLRAEDTAVYYCAKAGFTGGHFDIWGQGTLVTVSSASTKGPSVFPLAPSSKSTSGGTAALGCLVKDYFPEPVTVSWNSGALTSGVHTFPAVLQSSGLYSLSSVVTVPSSSLGTQTYICNVNHKPSNTKVDKKVEPKSCDKTHTCPPCPAPELLGGPSVFLFPPKPKDTLMISRTPEVTCVVVDVSHEDPEVKFNWYVDGVEVHNAKTKPREEQYNSTYRVVSVLTVLHQDWLNGKEYKCKVSNKALPAPIEKTISKAKGQPREPQVYTLPPSRDELTKNQVSLTCLVKGFYPSDIAVEWESNGQPENNYKTTPPVLDSDGSFFLYSKLTVDKSRWQQGNVFSCSVMHEALHNHYTQKSLSLSPGK

SEQ ID NO: 17 - protein, 214 aa, Artificial Sequence
  D11_IGG-L_AA
QSVLTQPPSASGTPGQRVTISCSGSSSNIGNNYVSWYQQLPGTAPKLLIYGNSNRPSGVPNRFSGSKSGTSASLAISGLRSEDEADYYCQSYDSSSWLFGGGTKLTVLGQPKAAPSVTLFPPSSEELQANKATLVCLISDFYPGAVTVAWKADSSPVKAGVETTTPSKQSNNKYAASSYLSLTPEQWKSHKSYSCQVTHEGSTVEKTVAPAECS

SEQ ID NO: 18 - DNA, 354 bp, Artificial Sequence
  D11_VH_NT
gaagtgcagctgctggaaagtggaggtggactggtgcagcctggcggcagcctgcgcctgagctgtgccgccagcggattcaccttcagcgattattattggacctgggttcgccaagcacctggcaaaggcctggaatgggtgagcggctcacctgtgtttggcgccgctaactatgcccagaactttcagggccgctttaccatcagccgcgataacagcaaaaacaccctgtatctgcagatgaacagcctgcgcgccgaggacaccgcagtctactactgtgccaaagccggctttaccggcggccattttgatatctggggacaaggtactctggtgaccgtgagcagc

SEQ ID NO: 19 - DNA, 324 bp, Artificial Sequence
  D11_VL_NT
cagagcgtgctgacccagcctcctagcgcctccggtacaccaggacagcgcgtgactattagctgtagcggcagcagcagcaacatcggcaacaactatgtgagctggtaccagcaactgcctggaactgcacctaagctgctgatctatggcaacagcaaccgccctagcggcgtgcctaatcgctttagcggtagcaaatcaggcaccagcgccagcctggccatcagcggtcttcgctccgaagatgaagccgattattattgtcagagctatgatagcagcagctggctgtttggtggcggtaccaagctgaccgtgctg

SEQ ID NO: 20 - DNA, 1344 bp, Artificial Sequence
  D11_IGG-H_NT
gaagtgcagctgctggaaagtggaggtggactggtgcagcctggcggcagcctgcgcctgagctgtgccgccagcggattcaccttcagcgattattattggacctgggttcgccaagcacctggcaaaggcctggaatgggtgagcggctcacctgtgtttggcgccgctaactatgcccagaactttcagggccgctttaccatcagccgcgataacagcaaaaacaccctgtatctgcagatgaacagcctgcgcgccgaggacaccgcagtctactactgtgccaaagccggctttaccggcggccattttgatatctggggacaaggtactctggtgaccgtgagcagcgctagcaccaagggcccatcggtcttccccctggcaccctcctccaagagcacctctgggggcacagcggccctgggctgcctggtcaaggactacttccccgaaccggtgacggtgtcgtggaactcaggcgccctgaccagcggcgtgcacaccttcccggctgtcctacagtcctcaggactctactccctcagcagcgtggtgaccgtgccctccagcagcttgggcacccagacctacatctgcaacgtgaatcacaagcccagcaacaccaaggtggacaagaaagttgagcccaaatcttgcgacaaaactcacacatgcccaccgtgcccagcacctgaactcctggggggaccgtcagtcttcctcttccccccaaaacccaaggacaccctcatgatctcccggacccctgaggtcacatgcgtggtggtggacgtgagccacgaagaccctgaggtcaagttcaactggtacgtggacggcgtggaggtgcataatgccaagacaaagccgcgggaggagcagtacaacagcacgtaccgtgtggtcagcgtcctcaccgtcctgcaccaggactggctgaatggcaaggagtacaagtgcaaggtctccaacaaagccctcccagcccccatcgagaaaaccatctccaaagccaaagggcagccccgagaaccacaggtgtacaccctgcccccatcccgggatgagctgaccaagaaccaggtcagcctgacctgcctggtcaaaggcttctatcccagcgacatcgccgtggagtgggagagcaatgggcagccggagaacaactacaagaccacgcctcccgtgctggactccgacggctccttcttcctctacagcaagctcaccgtggacaagagcaggtggcagcaggggaacgtcttctcatgctccgtgatgcatgaggctctgcacaaccactacacgcagaagagcctctccctgtccccgggtaaa

SEQ ID NO: 21 - DNA, 642 bp, Artificial Sequence
  D11_IGG-L_NT
cagagcgtgctgacccagcctcctagcgcctccggtacaccaggacagcgcgtgactattagctgtagcggcagcagcagcaacatcggcaacaactatgtgagctggtaccagcaactgcctggaactgcacctaagctgctgatctatggcaacagcaaccgccctagcggcgtgcctaatcgctttagcggtagcaaatcaggcaccagcgccagcctggccatcagcggtcttcgctccgaagatgaagccgattattattgtcagagctatgatagcagcagctggctgtttggtggcggtaccaagctgaccgtgctgggtcagcccaaggctgccccctcggtcacgctcttcccaccctcctctgaggagcttcaagccaacaaggccacactggtgtgtctcataagtgacttctacccgggagccgtgacagtggcctggaaggcagatagcagccccgtcaaggcgggagtggagaccaccacaccctccaaacaaagcaacaacaagtacgcggccagcagctacctgagcctgacgcctgagcagtggaagtcccacaaaagctacagctgccaggtcacgcatgaagggagcaccgtggagaagacagtggcccctgcagaatgctct

SEQ ID NO: 22 - protein, 117 aa, Artificial Sequence
  D11-B9_VH_AA
EVQLLESGGGLVQPGGSLRLSCAASGFTFSDYYWTWVRQAPGKGLEWVSGSPVFGAANYAQNFQGRFTISRDNSKNTLYLQMNSLRAEDTAVYYCAKAGIPGHFDIWGQGTLVTVSS

SEQ ID NO: 23 - protein, 108 aa, Artificial Sequence; identical to SEQ ID NO: 15
  D11-B9_VL_AA

SEQ ID NO: 24 - protein, 447 aa, Artificial Sequence
  D11-B9_IGG-H_AA
EVQLLESGGGLVQPGGSLRLSCAASGFTFSDYYWTWVRQAPGKGLEWVSGSPVFGAANYAQNFQGRFTISRDNSKNTLYLQMNSLRAEDTAVYYCAKAGIPGHFDIWGQGTLVTVSSASTKGPSVFPLAPSSKSTSGGTAALGCLVKDYFPEPVTVSWNSGALTSGVHTFPAVLQSSGLYSLSSVVTVPSSSLGTQTYICNVNHKPSNTKVDKKVEPKSCDKTHTCPPCPAPELLGGPSVFLFPPKPKDTLMISRTPEVTCVVVDVSHEDPEVKFNWYVDGVEVHNAKTKPREEQYNSTYRVVSVLTVLHQDWLNGKEYKCKVSNKALPAPIEKTISKAKGQPREPQVYTLPPSRDELTKNQVSLTCLVKGFYPSDIAVEWESNGQPENNYKTTPPVLDSDGSFFLYSKLTVDKSRWQQGNVFSCSVMHEALHNHYTQKSLSLSPGK

SEQ ID NO: 25 - protein, 214 aa, Artificial Sequence; identical to SEQ ID NO: 17
  D11-B9_IGG-L_AA

SEQ ID NO: 26 - DNA, 351 bp, Artificial Sequence
  D11-B9_VH_NT
gaagtgcagctgctggaaagtggaggtggactggtgcagcctggcggcagcctgcgcctgagctgtgccgccagcggattcaccttcagcgattattattggacctgggttcgccaagcacctggcaaaggcctggaatgggtgagcggctcacctgtgtttggcgccgctaactatgcccagaactttcagggccgctttaccatcagccgcgataacagcaaaaacaccctgtatctgcagatgaacagcctgcgcgccgaggacaccgcagtctactactgtgccaaagccggtattcctggccattttgatatctggggacaaggtactctggtgaccgtgagcagc

SEQ ID NO: 27 - DNA, 324 bp, Artificial Sequence; identical to SEQ ID NO: 19
  D11-B9_VL_NT

SEQ ID NO: 28 - DNA, 1341 bp, Artificial Sequence
  D11-B9_IGG-H_NT
gaagtgcagctgctggaaagtggaggtggactggtgcagcctggcggcagcctgcgcctgagctgtgccgccagcggattcaccttcagcgattattattggacctgggttcgccaagcacctggcaaaggcctggaatgggtgagcggctcacctgtgtttggcgccgctaactatgcccagaactttcagggccgctttaccatcagccgcgataacagcaaaaacaccctgtatctgcagatgaacagcctgcgcgccgaggacaccgcagtctactactgtgccaaagccggtattcctggccattttgatatctggggacaaggtactctggtgaccgtgagcagcgctagcaccaagggcccatcggtcttccccctggcaccctcctccaagagcacctctgggggcacagcggccctgggctgcctggtcaaggactacttccccgaaccggtgacggtgtcgtggaactcaggcgccctgaccagcggcgtgcacaccttcccggctgtcctacagtcctcaggactctactccctcagcagcgtggtgaccgtgccctccagcagcttgggcacccagacctacatctgcaacgtgaatcacaagcccagcaacaccaaggtggacaagaaagttgagcccaaatcttgcgacaaaactcacacatgcccaccgtgcccagcacctgaactcctggggggaccgtcagtcttcctcttccccccaaaacccaaggacaccctcatgatctcccggacccctgaggtcacatgcgtggtggtggacgtgagccacgaagaccctgaggtcaagttcaactggtacgtggacggcgtggaggtgcataatgccaagacaaagccgcgggaggagcagtacaacagcacgtaccgtgtggtcagcgtcctcaccgtcctgcaccaggactggctgaatggcaaggagtacaagtgcaaggtctccaacaaagccctcccagcccccatcgagaaaaccatctccaaagccaaagggcagccccgagaaccacaggtgtacaccctgcccccatcccgggatgagctgaccaagaaccaggtcagcctgacctgcctggtcaaaggcttctatcccagcgacatcgccgtggagtgggagagcaatgggcagccggagaacaactacaagaccacgcctcccgtgctggactccgacggctccttcttcctctacagcaagctcaccgtggacaagagcaggtggcagcaggggaacgtcttctcatgctccgtgatgcatgaggctctgcacaaccactacacgcagaagagcctctccctgtccccgggtaaa

SEQ ID NO: 29 - DNA, 642 bp, Artificial Sequence; identical to SEQ ID NO: 21
  D11-B9_IGG-L_NT